European Patent Specification EP 3 355 932 B1, published April 12, 2023. Title: OLIGONUCLEOTIDE CONJUGATION PROCESS. Applicant: Roche Innovation Center Copenhagen A/S. The sequence listing filed with the application follows.

SEQUENCE LISTING (4 sequences)

SEQ ID NO: 1 - DNA, 15 bp, Artificial
  Oligonucleotide nucleobase sequence
cagcgtaaagagagg

SEQ ID NO: 2 - DNA, 16 bp, Artificial
  Oligonucleotide nucleobase sequence
cagcgtaaagagaggt

SEQ ID NO: 3 - DNA, 15 bp, Artificial
  Oligonucleotide nucleobase sequence
cagcgtaaagagagg

SEQ ID NO: 4 - DNA, 12 bp, Artificial
  Oligonucleotide nucleobase sequence
gttgacactgtc